European Patent Application EP 4 420 729 A2, published August 28, 2024. Title: Antibody-drug conjugate formulations. Applicant: Genmab A/S. The sequence listing filed with the application follows.

SEQUENCE LISTING (80 sequences)

SEQ ID NO: 1 - protein, 119 aa, Homo sapiens
QVQLVESGGGVVQPGRSLRLSCVASGFTVSNDGMHWVRQAPGKGLEWVALIWYDGVNKNYADSVKGRFTISRDKSKNTLYLQMNSLRAEDTAVYYCARRPGTFYGLDVWGQGTTVTVSS

SEQ ID NO: 2 - protein, 8 aa, Homo sapiens
GFTVSNDG

SEQ ID NO: 3 - protein, 8 aa, Homo sapiens
IWYDGVNK

SEQ ID NO: 4 - protein, 12 aa, Homo sapiens
ARRPGTFYGLDV

SEQ ID NO: 5 - protein, 118 aa, Homo sapiens
EVQLLESGGGLVQPGGSLRLSCAASGFTFSNYAMSWVRQAPGKGLEWVSSISGSGDYTYYTDSVKGRFTISRDNSKNTLYLQMNSLRAEDTAVYYCARSPWGYYLDSWGQGTLVTVSS

SEQ ID NO: 6 - protein, 8 aa, Homo sapiens
GFTFSNYA

SEQ ID NO: 7 - protein, 8 aa, Homo sapiens
ISGSGDYT

SEQ ID NO: 8 - protein, 11 aa, Homo sapiens
ARSPWGYYLDS

SEQ ID NO: 9 - protein, 120 aa, Homo sapiens
EVQLLESGGGLVQPGGSLRLSCAASGFTFSSYAMSWVRQAPGKGLEWVSAISGSGDSTNYADSVKGRFTISRDNSKNTLYLQMNSLRAEDTAVYYCAKDGYFLLWYFDLWGRGTLVTVSS

SEQ ID NO: 10 - protein, 8 aa, Homo sapiens
GFTFSSYA

SEQ ID NO: 11 - protein, 8 aa, Homo sapiens
ISGSGDST

SEQ ID NO: 12 - protein, 13 aa, Homo sapiens
AKDGYFLLWYFDL

SEQ ID NO: 13 - protein, 118 aa, Homo sapiens
EVQLLESGGGLVQPGGSLRLSCAASGFTFSSYGMSWVRQAPGKGLEWVSVISGSGGTTYYADSVKGRFTISRDNSKNTLYLQMNSLRAEDTAVYYCAKAPWTYYFDYWGQGTLVTVSS

SEQ ID NO: 14 - protein, 8 aa, Homo sapiens
GFTFSSYG

SEQ ID NO: 15 - protein, 8 aa, Homo sapiens
ISGSGGTT

SEQ ID NO: 16 - protein, 11 aa, Homo sapiens
AKAPWTYYFDY

SEQ ID NO: 17 - protein, 118 aa, Homo sapiens
EVQLLESGGGLVQPGGSLRLSCAASGFTFNNYAMSWVRQAPGKGLEWVSSISGSGGRTYYADSVKGRFTISRDNSKNTLFLQMNSLRAEDTAVYYCAKTPWGYYFDYWGQGTLVTVSS

SEQ ID NO: 18 - protein, 8 aa, Homo sapiens
GFTFNNYA

SEQ ID NO: 19 - protein, 8 aa, Homo sapiens
ISGSGGRT

SEQ ID NO: 20 - protein, 11 aa, Homo sapiens
AKTPWGYYFDY

SEQ ID NO: 21 - protein, 118 aa, Homo sapiens
EVQLLESGGGLVQPGGSLRLSCAASGFTFSNYAMSWVRQAPAKGLDWVSGISGSGVTTYYADSVKGRFTISRDNSKDTLYLQMNSLRAEDTAVYFCAKTPWGYYFDYWGQGILVAVSS

SEQ ID NO: 22 - protein, 8 aa, Homo sapiens
GFTFSNYA

SEQ ID NO: 23 - protein, 8 aa, Homo sapiens
ISGSGVTT

SEQ ID NO: 24 - protein, 11 aa, Homo sapiens
AKTPWGYYFDY

SEQ ID NO: 25 - protein, 120 aa, Homo sapiens
QVQLVESGGGVVQPGRSLRLSCAASGFTFSRYAMHWVRQAPGKGLEWVAVISNDGYNDYYADSVKGRFTVSRDNSKNTLYLQMNSLRAEDTAVYYCARDGQLGRGYFDYWGQGTLVTVSS

SEQ ID NO: 26 - protein, 8 aa, Homo sapiens
GFTFSRYA

SEQ ID NO: 27 - protein, 8 aa, Homo sapiens
ISNDGYND

SEQ ID NO: 28 - protein, 13 aa, Homo sapiens
ARDGQLGRGYFDY

SEQ ID NO: 29 - protein, 120 aa, Homo sapiens
QVQLVESGGGVVQPGRSLRLSCPASGFTFSIYAMHWVRQAPGKGLEWVAVVSNDGYNKYYADSVKGRFTISRDNSKDTLYLQMNSLRAEDTAVYYCARDGQLGRGYFDYWGQGTLVTVSS

SEQ ID NO: 30 - protein, 8 aa, Homo sapiens
GFTFSIYA

SEQ ID NO: 31 - protein, 8 aa, Homo sapiens
VSNDGYNK

SEQ ID NO: 32 - protein, 13 aa, Homo sapiens
ARDGQLGRGYFDY

SEQ ID NO: 33 - protein, 118 aa, Homo sapiens
QVQLVQSGAEVRKPGSSVKVSCKASGGSFNNYPIFWVRQAPGQGFEWMGRIIPILGITAYAQKFQGRVTITADKSTSTAYMELNSLRSEDTAVYYCAGGDDLDAFDIWGQGTMVSVSS

SEQ ID NO: 34 - protein, 8 aa, Homo sapiens
GGSFNNYP

SEQ ID NO: 35 - protein, 8 aa, Homo sapiens
IIPILGIT

SEQ ID NO: 36 - protein, 11 aa, Homo sapiens
AGGDDLDAFDI

SEQ ID NO: 37 - protein, 120 aa, Homo sapiens
QVQLVESGGGVVQPGRSLRLSCAGSGFTFNRYAMYWVRQAPGKGLDWVAVISNDGINKYYADSVKGRFTISRDNSKNTLYLQMNSLRAEDTAVYYCARDHTMVRGAFDYWGQGTLVTVSS

SEQ ID NO: 38 - protein, 8 aa, Homo sapiens
GFTFNRYA

SEQ ID NO: 39 - protein, 8 aa, Homo sapiens
ISNDGINK

SEQ ID NO: 40 - protein, 13 aa, Homo sapiens
ARDHTMVRGAFDY

SEQ ID NO: 41 - protein, 107 aa, Homo sapiens
EIVLTQSPGTLSLSPGERATLSCRASQSVSSSYLAWYQQKPGQAPRLLIYGASSRATGIPDRFSGSGSGTDFTLTISRLEPEDFAVYYCQQYGSSLTFGGGTKVEIK

SEQ ID NO: 42 - protein, 7 aa, Homo sapiens
QSVSSSY

SEQ ID NO: 43 - skipped

SEQ ID NO: 44 - protein, 8 aa, Homo sapiens
QQYGSSLT

SEQ ID NO: 45 - protein, 107 aa, Homo sapiens
DIQMTQSPPSLSASAGDRVTITCRASQGISSRLAWYQQKPEKAPKSLIYAASSLQSGVPSRFSGSGSGTDFTLTISSLQPEDFATYYCQQYNSYPYTFGQGTKLEIK

SEQ ID NO: 46 - protein, 6 aa, Homo sapiens
QGISSR

SEQ ID NO: 47 - skipped

SEQ ID NO: 48 - protein, 9 aa, Homo sapiens
QQYNSYPYT

SEQ ID NO: 49 - protein, 108 aa, Homo sapiens
EIVLTQSPGTLSLSPGERATLSCRASQSVRSSYLAWYQQKPGQAPRLLIYGASSRATGIPDRFSGSGSGTDFTLTISRLEPEDFAVYYCQQYGSSPRTFGQGTKVEIK

SEQ ID NO: 50 - protein, 7 aa, Homo sapiens
QSVRSSY

SEQ ID NO: 51 - skipped

SEQ ID NO: 52 - protein, 9 aa, Homo sapiens
QQYGSSPRT

SEQ ID NO: 53 - protein, 108 aa, Homo sapiens
EIVLTQSPGTLSLSPGERATLSCRASQSVGSSSLAWYQQKPGQAPRLLIYGASSRATGIPDRFSGSGSGTDFTLTISRLEPEDFAVYYCQQYGSSPRTFGQGTKVEIK

SEQ ID NO: 54 - protein, 7 aa, Homo sapiens
QSVGSSS

SEQ ID NO: 55 - skipped

SEQ ID NO: 56 - protein, 9 aa, Homo sapiens
QQYGSSPRT

SEQ ID NO: 57 - protein, 107 aa, Homo sapiens
DIQMTQSPSSLSASVGDRVTITCRASQGISSRLAWYQQKPEKAPKSLIYAASSLQSGVPSRFSGSGSGTDFTLTISSLQPEDFATYYCQQYNSYPYTFGQGTKLEIK

SEQ ID NO: 58 - protein, 6 aa, Homo sapiens
QGISSR

SEQ ID NO: 59 - skipped

SEQ ID NO: 60 - protein, 9 aa, Homo sapiens
QQYNSYPYT

SEQ ID NO: 61 - protein, 108 aa, Homo sapiens
DIQMTQSPSSLSASVGDRVTITCRASQGISSWLAWYQQKPEKAPKSLIYAASSLQSGVPSRFSGSGSGTDFTLTISSLQPEDFATYYCQQYNSYPLYTFGQGTKLEIK

SEQ ID NO: 62 - protein, 6 aa, Homo sapiens
QGISSW

SEQ ID NO: 63 - skipped

SEQ ID NO: 64 - protein, 10 aa, Homo sapiens
QQYNSYPLYT

SEQ ID NO: 65 - protein, 107 aa, Homo sapiens
EIVLTQSPATLSLSPGERATLSCRASQSVSSYLAWYQQKPGQAPRLLIYDASNRATGIPARFSGSGSGTDFTLTISSLEPEDFAVYYCQQRSNWPLTFGGGTKVEIK

SEQ ID NO: 66 - protein, 6 aa, Homo sapiens
QSVSSY

SEQ ID NO: 67 - skipped

SEQ ID NO: 68 - protein, 9 aa, Homo sapiens
QQRSNWPLT

SEQ ID NO: 69 - protein, 107 aa, Homo sapiens
EIVLTQSPATLSLSPGERAILSCRASQSVSSYLAWYQQKPGQAPRLLIYDASNRATGIPARFSGSGSGTDFTLTISSLEPEDFAVYYCQQRSNWPLTFGGGTKVEIK

SEQ ID NO: 70 - protein, 6 aa, Homo sapiens
QSVSSY

SEQ ID NO: 71 - skipped

SEQ ID NO: 72 - protein, 9 aa, Homo sapiens
QQRSNWPLT

SEQ ID NO: 73 - protein, 107 aa, Homo sapiens
DIQMTQSPSSLSASVGDRVTITCRASQGISSWLAWYQQKPEKAPKSLIYAASSLQSGVPSRFSGSGSGTDFTLTISSLQPEDFATYYCQQYNSYPYTFGQGTKLEIK

SEQ ID NO: 74 - protein, 6 aa, Homo sapiens
QGISSW

SEQ ID NO: 75 - skipped

SEQ ID NO: 76 - protein, 9 aa, Homo sapiens
QQYNSYPYT

SEQ ID NO: 77 - protein, 107 aa, Homo sapiens; identical to SEQ ID NO: 65

SEQ ID NO: 78 - protein, 6 aa, Homo sapiens
QSVSSY

SEQ ID NO: 79 - skipped

SEQ ID NO: 80 - protein, 9 aa, Homo sapiens
QQRSNWPLT